European Patent Specification EP 3 377 633 B9, published October 4, 2023. Title: Recombinant Protein Production. Applicant: University of York. The sequence listing filed with the application follows.

SEQUENCE LISTING (10 sequences)

SEQ ID NO: 1 - DNA, 583 bp, Homo sapiens
ttagatctgcggccgcgtgagcagggtgcacttgctgcttttgtgccgctttaatgagttcacacagcagaatacctaaatctgcacagaaccttggttaacattttaaggtaggcaaacgcaggcataccaacttgttcctgttgccattgcagtgactaaaggagggatgtcacagggtattaattacagagcaggccatatgctatttttgtacagtaatcctttcctttttttccccatttttcttaaatcttaaaaataagactgaattctgatatcaagagttaaggtcccttcaatagttcagctggtagagcagaggactatagctacttcctcagtaggagacgtccttaggttgctggttcgattccagcttgaaggagacaagtacagttttggctgggcacggtggttcatggctgtaatcacagcactttgggaggttaaggcaggtggatcacgaggtcaggagatcaagatcatcctggccaatgtggtgaaactctgtctccggtgcgggtgccagggcgtgcccttgggctccccgggcgcgtactccacgcggccgcctcgagtt

SEQ ID NO: 2 - DNA, 21 bp, artificial sequence
  primer
gctggtagagcagaggactat

SEQ ID NO: 3 - DNA, 21 bp, artificial sequence
  primer
tcgaaccagcaacctaaggac

SEQ ID NO: 4 - DNA, 1003 bp, Homo sapiens
agatcttctagagtttaaaccgccgctcacagtacccgaaaggcgcatttttcacaaactgttgtagaaagagttcatggcggggtggcggcgggaaaaaaaaaaaaaaagctaacgccgtggccggtgcgggagtcgagcccgcgaccttggtgttatcagcaccacgctcttaccaactgagctaaccggccgcctgacggcacagtgcccctggagcgtataaaagggctccacgttcgcgcccgtccacgagcgattcctcgccaagcccgcgcgcctctggctgccttccgctttgccccagccgcggggactccggggaggagccaccgccccagcgctggccgggtttctcccgctcctccctgccaggctgtcctcgacaacctctgggccgagtccaagagatcccgcaagtcgctcctgcccgcatggggcttacagaacctgaaaggcgcattttgaaaaagagttgcagaaacagttcatggaagcttaagcttcgttcagcttcccttgggccccctggctgctcgggcccggatcgcggaccggggcgtttccggggatttctgaagcggacgaggggcagggcgggcgaaggccattcggctctccttctggctccagaatctcccaacccgcaggtgtgcagtgtgaccagcgcgactcaccgctctaatcgctccgattttccaaggccttgctcagtagtcctgccaggcgggctctgaggctggaagggattggggagttcggtgagtgcgccctgcctatagcgcccagtggaatcgctagtacctgtctctgtggcgcaatcggtcagagcgttcggctattaaccgaacggtgagtagttcaagaccacccagggacgcctgttctagctttttttaaagcattcatgtattatcatcactagagaatctccccctattcttcccatagtcctaagtccgaaaggttggttccaggccagcggcgcgccgctagcagatct

SEQ ID NO: 5 - DNA, 19 bp, Artificial Sequence
  primer
gctaacgccgtggccggtg

SEQ ID NO: 6 - DNA, 19 bp, Artificial Sequence
  primer
gctaacgccgtggccggtg

SEQ ID NO: 7 - DNA, 22 bp, Artificial Sequence
  primer
tcgctagtacctgtctctgtgg

SEQ ID NO: 8 - DNA, 22 bp, Artificial Sequence
  primer
cctgggtggtcttgaactactc

SEQ ID NO: 9 - DNA, 324 bp, Schizosaccharomyces pombe
ggatccttttcgttcaatcaagatattttatcacattatttcaaggttcaatgaatcattcgaagaatagtaacgaattcagatatattaaataaaggcacacataatctctaaagattacagtttaatggctctttcaaagtgtttagtaatatatacactaaatttctaaaattcagtagttatggcgaagtggccgagtggtctatggcgctagcttcaggtgaaagcaattgctagtctacgtatgtgggcgtgggttcgaaccccaccttcgtcaatataattttttatatcatgttaatggaattgagaaaaactagt

SEQ ID NO: 10 - DNA, 299 bp, Homo sapiens
gccgggcgcggtggcgcgtgcctgtagtcccagctactcgggaggctgaggctggaggatcgcttgagtccaggagttctgggctgtagtgcgctatgccgatcgggtgtccgcactaagttcggcatcaatatggtgacctcccgggagcgggggaccaccaggttgcctaaggaggggtgaaccggcccaggtcggaaacggagcaggtcaaaactcccgtgctgatcagtagtgggatcgcgcctgtgaatagccactgcactccagcctgggcaacatagcgagaccccgtctct